European Patent Application EP 4 501 963 A1, published February 5, 2025. Title: ANTI-HLA-G CHIMERIC ANTIGEN RECEPTORS AND USES THEREOF. Applicant: 에이치케이이노엔 주식회사. The sequence listing filed with the application follows.

SEQUENCE LISTING (48 sequences)

SEQ ID NO: 1 - DNA, 738 bp, Artificial Sequence
  source 1..738: mol_type = other DNA
gaagtacaactgctggaaagtggcgggggtctggttcagccgggaggctcacttaggttgtcatgtgcggcatccggatttacgttctccgattatgcgatgtcctgggttcggcaagctcctggtaaaggtttggagtgggtatccgtaatttctcatgatggaggcagtatctattatgccgatagcgtcaagggacgcttcactatttccagagacaattccaaaaataccctgtaccttcaaatgaactcactccgagccgaggacaccgcagtttactactgcgcgaaggggcctaggagaatcgcgaacgctattttcgattattggggtcaggggaccctggtgacggttagttctgggggtggaggcagtggaggcgggggtagtggaggagggggttcacaatttgtactgacccaacctccgtcagtctctgccgcccccggccaaaaagtaacgataagctgttcagggagcaactctaatataggcaactcttatgtctcttggtaccaacaagtacccggcgcagcgcctaggcttttgatatatgggtcaactaaccggccgagcggcgtgccagaccgcttttcaggtagtaagtcagggacgagtgccagtctggctatcaccggtctgcaagctgaggacgaggctgattattactgtcaaagctatgactcctcattgtccggctatgtttttggaacgggcacgaaggtaacagttcta

SEQ ID NO: 2 - protein, 246 aa, Artificial Sequence
EVQLLESGGGLVQPGGSLRLSCAASGFTFSDYAMSWVRQAPGKGLEWVSVISHDGGSIYYADSVKGRFTISRDNSKNTLYLQMNSLRAEDTAVYYCAKGPRRIANAIFDYWGQGTLVTVSSGGGGSGGGGSGGGGSQFVLTQPPSVSAAPGQKVTISCSGSNSNIGNSYVSWYQQVPGAAPRLLIYGSTNRPSGVPDRFSGSKSGTSASLAITGLQAEDEADYYCQSYDSSLSGYVFGTGTKVTVL

SEQ ID NO: 3 - DNA, 738 bp, Artificial Sequence
  source 1..738: mol_type = other DNA
gaggttcagttgcttgagtcaggcggaggactggttcaaccgggcggtagtttgaggctgagctgcgccgccagtggattcactttcagcgattacgcgatgtcctgggtccggcaggctccgggaaagggcctggagtgggtttctgtcataagccacgatggcgacagggtatattatgctgactcagtgaaaggtcgcttcacaatttctcgggacaactctaaaaataccctgtatttgcagatgaattctctcagagcggaggacaccgctgtttattattgtgcaaaaggcccccggaggatcgcgaatgccatattcgattactggggccaaggcacgcttgtaacggtttcatcaggtggaggagggagcggtggaggcgggtccggtggcggtggatctcagctcgtactcactcagcctccgtcagtatctggggccccgggtcaaaaggtcacaataagttgttccggttcttctagtaatatcgggcatagttatgtctcatggtaccagcagttgcctggaactgcaccaaagctcctgatatatggggataacaatcggcctagcggtgtacccgaccgctttagcggttctaaatcaggcacatctgcgtcccttgctattaccggactccaggccgaagacgaagcggactattactgtcagtcctacgacagttccttgtctgggtatgtgttcgggaccggaaccaaagtcactgtccta

SEQ ID NO: 4 - protein, 246 aa, Artificial Sequence
EVQLLESGGGLVQPGGSLRLSCAASGFTFSDYAMSWVRQAPGKGLEWVSVISHDGDRVYYADSVKGRFTISRDNSKNTLYLQMNSLRAEDTAVYYCAKGPRRIANAIFDYWGQGTLVTVSSGGGGSGGGGSGGGGSQLVLTQPPSVSGAPGQKVTISCSGSSSNIGHSYVSWYQQLPGTAPKLLIYGDNNRPSGVPDRFSGSKSGTSASLAITGLQAEDEADYYCQSYDSSLSGYVFGTGTKVTVL

SEQ ID NO: 5 - DNA, 738 bp, Artificial Sequence
  source 1..738: mol_type = other DNA
gaagtgcagcttttggaatctggcggcggactcgttcagccaggaggttcccttagactgtcatgcgcggctagcgggtttacgtttagcgactattcaatgtcttgggttcgacaggcaccgggcaaaggtctggagtgggtgagcgcaattagcccggatcggtctctggagtattacgccgactctgtgaaggggcgatttaccatcagccgggacaactccaaaaataccctgtatctgcaaatgaactcactgcgagcggaagacaccgcagtctactattgcgcaaaagggccacgccatctgacgaataatatatttgactattggggtcaaggtaccctcgtcacagttagctcaggtggcggcggttccggcggcggtggtagcggtgggggaggctcccaattcgtcttgacccagccaccaagcgtgagtgctgcccccggtcagaaggtcaccatatcttgtagtggctcaagttcaaacataggtcactcttatgtttcatggtatcaacaactccctggaacggcaccaaaacttttgatctatggtaacattcaccgaccgtccggagtacctgatagatttagcggttctacgtctgggacttccgcttctcttgctataacgggcttgcaggcggatgacgaggccgactactactgtggtgtgtgggattcttctctgtcagcggtagtgtttggaggcgggacaaaattgactgtacta

SEQ ID NO: 6 - protein, 246 aa, Artificial Sequence
EVQLLESGGGLVQPGGSLRLSCAASGFTFSDYSMSWVRQAPGKGLEWVSAISPDRSLEYYADSVKGRFTISRDNSKNTLYLQMNSLRAEDTAVYYCAKGPRHLTNNIFDYWGQGTLVTVSSGGGGSGGGGSGGGGSQFVLTQPPSVSAAPGQKVTISCSGSSSNIGHSYVSWYQQLPGTAPKLLIYGNIHRPSGVPDRFSGSTSGTSASLAITGLQADDEADYYCGVWDSSLSAVVFGGGTKLTVL

SEQ ID NO: 7 - DNA, 63 bp, Artificial Sequence
  source 1..63: mol_type = other DNA
atggccttaccagtgaccgccttgctcctgccgctggccttgctgctccacgccgccaggccg

SEQ ID NO: 8 - protein, 21 aa, Artificial Sequence
MALPVTALLLPLALLLHAARP

SEQ ID NO: 9 - DNA, 135 bp, Artificial Sequence
  source 1..135: mol_type = other DNA
accacgacgccagcgccgcgaccaccaacaccggcgcccaccatcgcgtcgcagcccctgtccctgcgcccagaggcgtgccggccagcggcggggggcgcagtgcacacgagggggctggacttcgcctgtgat

SEQ ID NO: 10 - protein, 45 aa, Artificial Sequence
TTTPAPRPPTPAPTIASQPLSLRPEACRPAAGGAVHTRGLDFACD

SEQ ID NO: 11 - DNA, 72 bp, Artificial Sequence
  source 1..72: mol_type = other DNA
atctacatctgggcgcccttggccgggacttgtggggtccttctcctgtcactggttatcaccctttactgc

SEQ ID NO: 12 - protein, 24 aa, Artificial Sequence
IYIWAPLAGTCGVLLLSLVITLYC

SEQ ID NO: 13 - DNA, 126 bp, Artificial Sequence
  source 1..126: mol_type = other DNA
aaacggggcagaaagaaactcctgtatatattcaaacaaccatttatgagaccagtacaaactactcaagaggaagatggctgtagctgccgatttccagaagaagaagaaggaggatgtgaactg

SEQ ID NO: 14 - protein, 42 aa, Artificial Sequence
KRGRKKLLYIFKQPFMRPVQTTQEEDGCSCRFPEEEEGGCEL

SEQ ID NO: 15 - DNA, 336 bp, Artificial Sequence
  source 1..336: mol_type = other DNA
agagtgaagttcagcaggagcgcagacgcccccgcgtacaagcagggccagaaccagctctataacgagctcaatctaggacgaagagaggagtacgatgttttggacaagagacgtggccgggaccctgagatggggggaaagccgagaaggaagaaccctcaggaaggcctgtacaatgaactgcagaaagataagatggcggaggcctacagtgagattgggatgaaaggcgagcgccggaggggcaaggggcacgatggcctttaccagggtctcagtacagccaccaaggacacctacgacgcccttcacatgcaggccctgccccctcgc

SEQ ID NO: 16 - protein, 112 aa, Artificial Sequence
RVKFSRSADAPAYKQGQNQLYNELNLGRREEYDVLDKRRGRDPEMGGKPRRKNPQEGLYNELQKDKMAEAYSEIGMKGERRRGKGHDGLYQGLSTATKDTYDALHMQALPPR

SEQ ID NO: 17 - DNA, 1473 bp, Artificial Sequence
  source 1..1473: mol_type = other DNA
atggccttaccagtgaccgccttgctcctgccgctggccttgctgctccacgccgccaggccggaagtacaactgctggaaagtggcgggggtctggttcagccgggaggctcacttaggttgtcatgtgcggcatccggatttacgttctccgattatgcgatgtcctgggttcggcaagctcctggtaaaggtttggagtgggtatccgtaatttctcatgatggaggcagtatctattatgccgatagcgtcaagggacgcttcactatttccagagacaattccaaaaataccctgtaccttcaaatgaactcactccgagccgaggacaccgcagtttactactgcgcgaaggggcctaggagaatcgcgaacgctattttcgattattggggtcaggggaccctggtgacggttagttctgggggtggaggcagtggaggcgggggtagtggaggagggggttcacaatttgtactgacccaacctccgtcagtctctgccgcccccggccaaaaagtaacgataagctgttcagggagcaactctaatataggcaactcttatgtctcttggtaccaacaagtacccggcgcagcgcctaggcttttgatatatgggtcaactaaccggccgagcggcgtgccagaccgcttttcaggtagtaagtcagggacgagtgccagtctggctatcaccggtctgcaagctgaggacgaggctgattattactgtcaaagctatgactcctcattgtccggctatgtttttggaacgggcacgaaggtaacagttctaaccacgacgccagcgccgcgaccaccaacaccggcgcccaccatcgcgtcgcagcccctgtccctgcgcccagaggcgtgccggccagcggcggggggcgcagtgcacacgagggggctggacttcgcctgtgatatctacatctgggcgcccttggccgggacttgtggggtccttctcctgtcactggttatcaccctttactgcaaacggggcagaaagaaactcctgtatatattcaaacaaccatttatgagaccagtacaaactactcaagaggaagatggctgtagctgccgatttccagaagaagaagaaggaggatgtgaactgagagtgaagttcagcaggagcgcagacgcccccgcgtacaagcagggccagaaccagctctataacgagctcaatctaggacgaagagaggagtacgatgttttggacaagagacgtggccgggaccctgagatggggggaaagccgagaaggaagaaccctcaggaaggcctgtacaatgaactgcagaaagataagatggcggaggcctacagtgagattgggatgaaaggcgagcgccggaggggcaaggggcacgatggcctttaccagggtctcagtacagccaccaaggacacctacgacgcccttcacatgcaggccctgccccctcgctaa

SEQ ID NO: 18 - protein, 490 aa, Artificial Sequence
MALPVTALLLPLALLLHAARPEVQLLESGGGLVQPGGSLRLSCAASGFTFSDYAMSWVRQAPGKGLEWVSVISHDGGSIYYADSVKGRFTISRDNSKNTLYLQMNSLRAEDTAVYYCAKGPRRIANAIFDYWGQGTLVTVSSGGGGSGGGGSGGGGSQFVLTQPPSVSAAPGQKVTISCSGSNSNIGNSYVSWYQQVPGAAPRLLIYGSTNRPSGVPDRFSGSKSGTSASLAITGLQAEDEADYYCQSYDSSLSGYVFGTGTKVTVLTTTPAPRPPTPAPTIASQPLSLRPEACRPAAGGAVHTRGLDFACDIYIWAPLAGTCGVLLLSLVITLYCKRGRKKLLYIFKQPFMRPVQTTQEEDGCSCRFPEEEEGGCELRVKFSRSADAPAYKQGQNQLYNELNLGRREEYDVLDKRRGRDPEMGGKPRRKNPQEGLYNELQKDKMAEAYSEIGMKGERRRGKGHDGLYQGLSTATKDTYDALHMQALPPR

SEQ ID NO: 19 - DNA, 1473 bp, Artificial Sequence
  source 1..1473: mol_type = other DNA
atggccttaccagtgaccgccttgctcctgccgctggccttgctgctccacgccgccaggccggaggttcagttgcttgagtcaggcggaggactggttcaaccgggcggtagtttgaggctgagctgcgccgccagtggattcactttcagcgattacgcgatgtcctgggtccggcaggctccgggaaagggcctggagtgggtttctgtcataagccacgatggcgacagggtatattatgctgactcagtgaaaggtcgcttcacaatttctcgggacaactctaaaaataccctgtatttgcagatgaattctctcagagcggaggacaccgctgtttattattgtgcaaaaggcccccggaggatcgcgaatgccatattcgattactggggccaaggcacgcttgtaacggtttcatcaggtggaggagggagcggtggaggcgggtccggtggcggtggatctcagctcgtactcactcagcctccgtcagtatctggggccccgggtcaaaaggtcacaataagttgttccggttcttctagtaatatcgggcatagttatgtctcatggtaccagcagttgcctggaactgcaccaaagctcctgatatatggggataacaatcggcctagcggtgtacccgaccgctttagcggttctaaatcaggcacatctgcgtcccttgctattaccggactccaggccgaagacgaagcggactattactgtcagtcctacgacagttccttgtctgggtatgtgttcgggaccggaaccaaagtcactgtcctaaccacgacgccagcgccgcgaccaccaacaccggcgcccaccatcgcgtcgcagcccctgtccctgcgcccagaggcgtgccggccagcggcggggggcgcagtgcacacgagggggctggacttcgcctgtgatatctacatctgggcgcccttggccgggacttgtggggtccttctcctgtcactggttatcaccctttactgcaaacggggcagaaagaaactcctgtatatattcaaacaaccatttatgagaccagtacaaactactcaagaggaagatggctgtagctgccgatttccagaagaagaagaaggaggatgtgaactgagagtgaagttcagcaggagcgcagacgcccccgcgtacaagcagggccagaaccagctctataacgagctcaatctaggacgaagagaggagtacgatgttttggacaagagacgtggccgggaccctgagatggggggaaagccgagaaggaagaaccctcaggaaggcctgtacaatgaactgcagaaagataagatggcggaggcctacagtgagattgggatgaaaggcgagcgccggaggggcaaggggcacgatggcctttaccagggtctcagtacagccaccaaggacacctacgacgcccttcacatgcaggccctgccccctcgctaa

SEQ ID NO: 20 - protein, 490 aa, Artificial Sequence
MALPVTALLLPLALLLHAARPEVQLLESGGGLVQPGGSLRLSCAASGFTFSDYAMSWVRQAPGKGLEWVSVISHDGDRVYYADSVKGRFTISRDNSKNTLYLQMNSLRAEDTAVYYCAKGPRRIANAIFDYWGQGTLVTVSSGGGGSGGGGSGGGGSQLVLTQPPSVSGAPGQKVTISCSGSSSNIGHSYVSWYQQLPGTAPKLLIYGDNNRPSGVPDRFSGSKSGTSASLAITGLQAEDEADYYCQSYDSSLSGYVFGTGTKVTVLTTTPAPRPPTPAPTIASQPLSLRPEACRPAAGGAVHTRGLDFACDIYIWAPLAGTCGVLLLSLVITLYCKRGRKKLLYIFKQPFMRPVQTTQEEDGCSCRFPEEEEGGCELRVKFSRSADAPAYKQGQNQLYNELNLGRREEYDVLDKRRGRDPEMGGKPRRKNPQEGLYNELQKDKMAEAYSEIGMKGERRRGKGHDGLYQGLSTATKDTYDALHMQALPPR

SEQ ID NO: 21 - DNA, 1473 bp, Artificial Sequence
  source 1..1473: mol_type = other DNA
atggccttaccagtgaccgccttgctcctgccgctggccttgctgctccacgccgccaggccggaagtgcagcttttggaatctggcggcggactcgttcagccaggaggttcccttagactgtcatgcgcggctagcgggtttacgtttagcgactattcaatgtcttgggttcgacaggcaccgggcaaaggtctggagtgggtgagcgcaattagcccggatcggtctctggagtattacgccgactctgtgaaggggcgatttaccatcagccgggacaactccaaaaataccctgtatctgcaaatgaactcactgcgagcggaagacaccgcagtctactattgcgcaaaagggccacgccatctgacgaataatatatttgactattggggtcaaggtaccctcgtcacagttagctcaggtggcggcggttccggcggcggtggtagcggtgggggaggctcccaattcgtcttgacccagccaccaagcgtgagtgctgcccccggtcagaaggtcaccatatcttgtagtggctcaagttcaaacataggtcactcttatgtttcatggtatcaacaactccctggaacggcaccaaaacttttgatctatggtaacattcaccgaccgtccggagtacctgatagatttagcggttctacgtctgggacttccgcttctcttgctataacgggcttgcaggcggatgacgaggccgactactactgtggtgtgtgggattcttctctgtcagcggtagtgtttggaggcgggacaaaattgactgtactaaccacgacgccagcgccgcgaccaccaacaccggcgcccaccatcgcgtcgcagcccctgtccctgcgcccagaggcgtgccggccagcggcggggggcgcagtgcacacgagggggctggacttcgcctgtgatatctacatctgggcgcccttggccgggacttgtggggtccttctcctgtcactggttatcaccctttactgcaaacggggcagaaagaaactcctgtatatattcaaacaaccatttatgagaccagtacaaactactcaagaggaagatggctgtagctgccgatttccagaagaagaagaaggaggatgtgaactgagagtgaagttcagcaggagcgcagacgcccccgcgtacaagcagggccagaaccagctctataacgagctcaatctaggacgaagagaggagtacgatgttttggacaagagacgtggccgggaccctgagatggggggaaagccgagaaggaagaaccctcaggaaggcctgtacaatgaactgcagaaagataagatggcggaggcctacagtgagattgggatgaaaggcgagcgccggaggggcaaggggcacgatggcctttaccagggtctcagtacagccaccaaggacacctacgacgcccttcacatgcaggccctgccccctcgctaa

SEQ ID NO: 22 - protein, 490 aa, Artificial Sequence
MALPVTALLLPLALLLHAARPEVQLLESGGGLVQPGGSLRLSCAASGFTFSDYSMSWVRQAPGKGLEWVSAISPDRSLEYYADSVKGRFTISRDNSKNTLYLQMNSLRAEDTAVYYCAKGPRHLTNNIFDYWGQGTLVTVSSGGGGSGGGGSGGGGSQFVLTQPPSVSAAPGQKVTISCSGSSSNIGHSYVSWYQQLPGTAPKLLIYGNIHRPSGVPDRFSGSTSGTSASLAITGLQADDEADYYCGVWDSSLSAVVFGGGTKLTVLTTTPAPRPPTPAPTIASQPLSLRPEACRPAAGGAVHTRGLDFACDIYIWAPLAGTCGVLLLSLVITLYCKRGRKKLLYIFKQPFMRPVQTTQEEDGCSCRFPEEEEGGCELRVKFSRSADAPAYKQGQNQLYNELNLGRREEYDVLDKRRGRDPEMGGKPRRKNPQEGLYNELQKDKMAEAYSEIGMKGERRRGKGHDGLYQGLSTATKDTYDALHMQALPPR

SEQ ID NO: 23 - DNA, 45 bp, Artificial Sequence
  source 1..45: mol_type = other DNA
gggggtggaggcagtggaggcgggggtagtggaggagggggttca

SEQ ID NO: 24 - protein, 15 aa, Artificial Sequence
GGGGSGGGGSGGGGS

SEQ ID NO: 25 - protein, 121 aa, Artificial Sequence
EVQLLESGGGLVQPGGSLRLSCAASGFTFSDYAMSWVRQAPGKGLEWVSVISHDGGSIYYADSVKGRFTISRDNSKNTLYLQMNSLRAEDTAVYYCAKGPRRIANAIFDYWGQGTLVTVSS

SEQ ID NO: 26 - protein, 110 aa, Artificial Sequence
QFVLTQPPSVSAAPGQKVTISCSGSNSNIGNSYVSWYQQVPGAAPRLLIYGSTNRPSGVPDRFSGSKSGTSASLAITGLQAEDEADYYCQSYDSSLSGYVFGTGTKVTVL

SEQ ID NO: 27 - protein, 121 aa, Artificial Sequence
EVQLLESGGGLVQPGGSLRLSCAASGFTFSDYAMSWVRQAPGKGLEWVSVISHDGDRVYYADSVKGRFTISRDNSKNTLYLQMNSLRAEDTAVYYCAKGPRRIANAIFDYWGQGTLVTVSS

SEQ ID NO: 28 - protein, 110 aa, Artificial Sequence
QLVLTQPPSVSGAPGQKVTISCSGSSSNIGHSYVSWYQQLPGTAPKLLIYGDNNRPSGVPDRFSGSKSGTSASLAITGLQAEDEADYYCQSYDSSLSGYVFGTGTKVTVL

SEQ ID NO: 29 - protein, 121 aa, Artificial Sequence
EVQLLESGGGLVQPGGSLRLSCAASGFTFSDYSMSWVRQAPGKGLEWVSAISPDRSLEYYADSVKGRFTISRDNSKNTLYLQMNSLRAEDTAVYYCAKGPRHLTNNIFDYWGQGTLVTVSS

SEQ ID NO: 30 - protein, 110 aa, Artificial Sequence
QFVLTQPPSVSAAPGQKVTISCSGSSSNIGHSYVSWYQQLPGTAPKLLIYGNIHRPSGVPDRFSGSTSGTSASLAITGLQADDEADYYCGVWDSSLSAVVFGGGTKLTVL

SEQ ID NO: 31 - protein, 5 aa, Artificial Sequence
DYAMS

SEQ ID NO: 32 - protein, 17 aa, Artificial Sequence
VISHDGGSIYYADSVKG

SEQ ID NO: 33 - protein, 12 aa, Artificial Sequence
GPRRIANAIFDY

SEQ ID NO: 34 - protein, 13 aa, Artificial Sequence
SGSNSNIGNSYVS

SEQ ID NO: 35 - protein, 7 aa, Artificial Sequence
GSTNRPS

SEQ ID NO: 36 - protein, 11 aa, Artificial Sequence
QSYDSSLSGYV

SEQ ID NO: 37 - protein, 5 aa, Artificial Sequence
DYAMS

SEQ ID NO: 38 - protein, 17 aa, Artificial Sequence
VISHDGDRVYYADSVKG

SEQ ID NO: 39 - protein, 12 aa, Artificial Sequence
GPRRIANAIFDY

SEQ ID NO: 40 - protein, 13 aa, Artificial Sequence
SGSSSNIGHSYVS

SEQ ID NO: 41 - protein, 7 aa, Artificial Sequence
GDNNRPS

SEQ ID NO: 42 - protein, 11 aa, Artificial Sequence
QSYDSSLSGYV

SEQ ID NO: 43 - protein, 5 aa, Artificial Sequence
DYSMS

SEQ ID NO: 44 - protein, 17 aa, Artificial Sequence
AISPDRSLEYYADSVKG

SEQ ID NO: 45 - protein, 12 aa, Artificial Sequence
GPRHLTNNIFDY

SEQ ID NO: 46 - protein, 13 aa, Artificial Sequence
SGSSSNIGHSYVS

SEQ ID NO: 47 - protein, 7 aa, Artificial Sequence
GNIHRPS

SEQ ID NO: 48 - protein, 11 aa, Artificial Sequence
GVWDSSLSAVV